European Patent Application EP 4 729 543 A1, published April 22, 2026. Title: ANTI-IL-4 RECEPTOR ANTIBODIES FOR VETERINARY USE. Applicant: Harfang Therapeutics. The sequence listing filed with the application follows.

SEQUENCE LISTING (24 sequences)

SEQ ID NO: 1 - protein, 8 aa, synthetic construct
GFTFSSYG

SEQ ID NO: 2 - protein, 8 aa, synthetic construct
GFTFSDYG

SEQ ID NO: 3 - protein, 8 aa, synthetic construct
GFTFTDYS

SEQ ID NO: 4 - protein, 8 aa, synthetic construct
IRHDGTVT

SEQ ID NO: 5 - protein, 8 aa, synthetic construct
ISRSGSIT

SEQ ID NO: 6 - protein, 8 aa, synthetic construct
INIGGSNT

SEQ ID NO: 7 - protein, 7 aa, synthetic construct
ANSRFDY

SEQ ID NO: 8 - protein, 9 aa, synthetic construct
ARGIGTLDY

SEQ ID NO: 9 - protein, 10 aa, synthetic construct
AAGFSDSLRY

SEQ ID NO: 10 - protein, 8 aa, synthetic construct
SSNIGGFN

SEQ ID NO: 11 - protein, 7 aa, synthetic construct
SEHSNYI

SEQ ID NO: 12 - protein, 9 aa, synthetic construct
SSNVGYGDY

SEQ ID NO: 13 - skipped

SEQ ID NO: 14 - protein, 7 aa, synthetic construct
VRSDGSY

SEQ ID NO: 15 - skipped

SEQ ID NO: 16 - protein, 11 aa, synthetic construct
STWDNSLKVGV

SEQ ID NO: 17 - protein, 13 aa, synthetic construct
GTDYKISGQYGHV

SEQ ID NO: 18 - protein, 11 aa, synthetic construct
SSYENSRSNSV

SEQ ID NO: 19 - protein, 114 aa, synthetic construct
EVQLVESGGDLVTPGGSLTLSCVASGFTFSSYGMSWVRQSPGKGLQWVAWIRHDGTVTYYADAVKGRFTISRDNAKNTLYLQMNSLRAEDTAVYYCANSRFDYWGQGTLVTVSS

SEQ ID NO: 20 - protein, 116 aa, synthetic construct
GVQLVESGGDLVKPGGSLRLSCVASGFTFSDYGMTWVRQSPGKGLQWVAGISRSGSITYYTDAVKGRFTISRDNAKNTLYLQMNSLRAEDTAVYYCARGIGTLDYWGQGTLVTISS

SEQ ID NO: 21 - protein, 117 aa, synthetic construct
EVQLVESGGDLVKPGGSLRLACVASGFTFTDYSMQWVRQAPGKGLQWVAYINIGGSNTNYADTVKGRFTISRDNAKNTLYLQMNSLRAEDTAVYYCAAGFSDSLRYWGQGTLVTVSS

SEQ ID NO: 22 - protein, 110 aa, synthetic construct
QAVLNQPASVTGSLGQRVTISCTGSSSNIGGFNVGWFQQFPGTGPRTVIYNTSNRPSGVSDRFSGSKSGSTATLTISGLQAEDEADYYCSTWDNSLKVGVFGGGTHLTVL

SEQ ID NO: 23 - protein, 116 aa, synthetic construct
LPVLTQPTNASASLEESVKLTCTLSSEHSNYIVQWYQQQPGKAPRYLMYVRSDGSYKRGDGIPSRFSGSSSGADRYLTISNIKSEDEDDYYYCGTDYKISGQYGHVFGSGTHLTVL

SEQ ID NO: 24 - protein, 111 aa, synthetic construct
QAVLTQPASVSGSLGQRVTISCTGSSSNVGYGDYVGWYQQLPGTSPRTLIFDSSRRPSGVPDRFSGSRSGTTATLTISGLQAEDEADYYCSSYENSRSNSVFGGGTQLTVL